European Patent Application EP 4 545 635 A1, published April 30, 2025. Title: RECOMBINANT ONCOLYTIC VIRUS AND USE THEREOF. Applicant: JOINT BIOSCIENCES (SH) LTD. Application EP. The sequence listing filed with the application follows.

SEQUENCE LISTING (41 sequences)

SEQ ID NO: 1 - protein, 229 aa, Vesicular Stomatitis Virus
MSSLKKILGLKGKGKKSKKLGIAPPPYEEDTNMEYAPSAPIDKSYFGVNEMDTHDPNQLRYEKFFFTVKMTVRSNRPFRTYSDVAAAVSHWDHMYIGMAGKRPFYKILAFLGSSNLKATPAVLADQGQPEYHAHCEGRAYLPHRMGKTPPMLNVPEHFRRPFNIGLYKGTIELTMTIYDDESLEAAPMIWDHFNSSKFSDFREKALMFGLIVEKKASGAWVLDSVSHFK

SEQ ID NO: 2 - protein, 229 aa, synthetic construct
MSSLKKILGLKGKGKKSKKLGIAPPPYEEDTNMEYAPSAPIDKSYFGVNERDTHDPNQLRYEKFFFTVKMTVRSNRPFRTYSDVAAAVSHWDHMYIGMAGKRPFYKILAFLGSSNLKATPAVLADQGQPEYHAHCEGRAYLPHRMGKTPPMLNVPEHFRRPFNIGLYKGTIELTMTIYDDESLEAAPMIWDHFNSSKFSDFREKALMFGLIVEKKASGAWFLDSVRHFK

SEQ ID NO: 3 - protein, 229 aa, synthetic construct
MSSLKKILGLKGKGKKSKKLGIAPPPYEEDTSMEYAPSAPIDKSYFGVDERDTYDPNQLRYEKFFFTVKMTVRSNRPFRTYSDVAAAVSHWDHMYIGMAGKRPFYKILAFLGSSNLKATPAVLADQGQPEYHAHCEGRAYLPHRMGKTPPMLNVPEHFRRPFNIGLYKGTIELTMTIYDDESLEAAPMIWDHFNSSKFSDFREKALMFGLIVEKKASGAWFLDSIRHFK

SEQ ID NO: 4 - protein, 228 aa, synthetic construct
MSSLKKILGLKGKGKKSKKLGIAPPPYEEDTSMEYAPSAPIDKSYFGVDERDTYDPNQLRYEKFFFTVKMTVRSNRPFRTYSDVAAAVSHWDHMYIGMAGKRPFYKILAFGSSNLKATPAVLADQGQPEYHAHCEGRAYLPHRMGKTPPMLNVPEHFRRPFNIGLYKGTIELTMTIYDDESLEAAPMIWDHFNSSKFSDFREKALMFGLIVEKKASGAWFLDSIRHFK

SEQ ID NO: 5 - protein, 229 aa, synthetic construct
MSSLKKILGLKGKGKKSKKLGIAPPPYEEDTSMEYAPSAPIDKSYFGVDERDTYDPNQLRYEKFFFTVKMTVRSNRPFRTYSDVAAAVSHWDHMYIGMAGKRPFYKILAFAGSSNLKATPAVLADQGQPEYHAHCEGRAYLPHRMGKTPPMLNVPEHFRRPFNIGLYKGTIELTMTIYDDESLEAAPMIWDHFNSSKFSDFREKALMFGLIVEKKASGAWFLDSIRHFK

SEQ ID NO: 6 - protein, 229 aa, synthetic construct
MSSLKKILGLKGKGKKSKKLEIAPPPYEEDTSMEYAPSAPIDKSYFGVDERDTYDPNQLRYEKFFFTVKMTVRSNRPFRTYSDVAAAVSHWDHMYIGMAGKRPFYKILAFLGSSNLKATPAVLADQGQPEYHAHCEGRAYLPHRMGKTPPMLNVPEHFRRPFNIGLYKGTIELTMTIYDDESLEAAPMIWDHFNSSKFSDFREKALMFGLIVEKKASGAWFLDSIRHFK

SEQ ID NO: 7 - protein, 229 aa, synthetic construct
MSSLKKILGLKGKGKKSKKLEIAPPPYEEDTSAEYAPSAPIDKSYFGVDERDTYDPNQLRYEKFFFTVKMTVRSNRPFRTYSDVAAAVSHWDHMYIGMAGKRPFYKILAFLGSSNLKATPAVLADQGQPEYHAHCEGRAYLPHRMGKTPPMLNVPEHFRRPFNIGLYKGTIELTMTIYDDESLEAAPMIWDHFNSSKFSDFREKALMFGLIVEKKASGAWFLDSIRHFK

SEQ ID NO: 8 - protein, 229 aa, synthetic construct
MSSLKKILGLKGKGKKSKKLEIAPPPYEEDTSAEYAPSAPIDKSYFGVDERDTYDPNQLRYEKFFFTVKMTVRSNRPFRTYSDVAAAVSHWDHMYIGMAGKRPFYKILAFLGSSNLKATPAVLADQGQPEYHTHCEGRAYLPHRMGKTPPMLNVPEHFRRPFNIGLYKGTIELTMTIYDDESLEAAPMIWDHFNSSKFSDFREKALMFGLIVEKKASGAWFLDSIRHFK

SEQ ID NO: 9 - protein, 229 aa, synthetic construct
MSSLKKILGLKGKGKKSKKLGIAPPPYEEDTSAEYAPSAPIDKSYFGVDERDTYDPNQLRYEKFFFTVKMTVRSNRPFRTYSDVAAAVSHWDHMYIGMAGKRPFYKILAFLGSSNLKATPAVLADQGQPEYHAHCEGRAYLPHRMGKTPPMLNVPEHFRRPFNIGLYKGTIELTMTIYDDESLEAAPMIWDHFNSSKFSDFREKALMFGLIVEKKASGAWFLDSIRHFK

SEQ ID NO: 10 - protein, 229 aa, synthetic construct
MSSLKKILGLKGKGKKSKKLGIAPPPYEEDTSAEYAPSAPIDKSYFGVDERDTYDPNQLRYEKFFFTVKMTVRSNRPFRTYSDVAAAVSHWDHMYIGMAGKRPFYKILAFLGSSNLKATPAVLADQGQPEYHTHCEGRAYLPHRMGKTPPMLNVPEHFRRPFNIGLYKGTIELTMTIYDDESLEAAPMIWDHFNSSKFSDFREKALMFGLIVEKKASGAWFLDSIRHFK

SEQ ID NO: 11 - protein, 229 aa, synthetic construct
MSSLKKILGLKGKGKKSKKLGIAPPPYEEDTSMEYAPSAPIDKSYFGVDERDTYDPNQLRYEKFFFTVKMTVRSNRPFRTYSDVAAAVSHWDHMYIGMAGKRPFYKILAFLGSSNLKATPAVLADQGQPEYHTHCEGRAYLPHRMGKTPPMLNVPEHFRRPFNIGLYKGTIELTMTIYDDESLEAAPMIWDHFNSSKFSDFREKALMFGLIVEKKASGAWFLDSIRHFK

SEQ ID NO: 12 - protein, 511 aa, Vesicular Stomatitis Virus
MKCLLYLAFLFIGVNCKFTIVFPHNQKGNWKNVPSNYHYCPSSSDLNWHNDLVGTALQVKMPKSHKAIQADGWMCHASKWVTTCDFRWYGPKYITHSIRSFTPSVEQCKESIEQTKQGTWLNPGFPPQSCGYATVTDAEAAIVQVTPHHVLVDEYTGEWVDSQFINGKCSNDICPTVHNSTTWHSDYKVKGLCDSNLISMDITFFSEDGELSSLGKKGTGFRSNYFAYETGDKACKMQYCKHWGVRLPSGVWFEMADKDLFAAARFPECPEGSSISAPSQTSVDVSLIQDVERILDYSLCQETWSKIRAGLPISPVDLSYLAPKNPGTGPVFTIINGTLKYFETRYIRVDIAAPILSRMVGMISGTTTERVLWDDWAPYEDVEIGPNGVLRTSSGYKFPLYMIGHGMLDSDLHLSSKAQVFEHPHIQDAASQLPDGETLFFGDTGLSKNPIEFVEGWFSSWKSSIASFFFTIGLIIGLFLVLRVGIYLCIKLKHTKKRQIYTDIEMNRLGK

SEQ ID NO: 13 - protein, 511 aa, synthetic construct
MKCLLYLAFLFIGVNCKFTIVFPHNQKGNWKNVPSNYHYCPSSSDLNWHNDLIGTALQVKMPKSHKAIQADGWMCHASKWVTTCDFRWYGPKYITHSIRSFTPSVEQCKESIEQTKQGTWLNPGFPPQSCGYATVTDAEAVIVQVTPHHVLVDEYTGEWVDSQFINGKCSNYICPTVHNSTTWHSDYKVKGLCDSNLISMDITFFSEDGELSSLGKEGTGFRSNYFAYETGGKACKMQYCKHWGVRLPSGVWFEMADKDLFAAARFPECPEGSSISAPSQTSVDVSLIQDVERILDYSLCQETWSKIRAGLPISPVDLSYLAPKNPGTGPAFTIINGTLKYFETRYIRVDIAAPILSRMVGMISGTTTERELWDDWAPYEDVEIGPNGVLRTSSGYKFPLYMIGHGMLDSDLHLSSKAQVFEHPHIQDAASQLPDDESLFFGDTGLSKNPIELVEGWFSSWKSSIASFFFIIGLIIGLFLVLRVGIHLCIKLKHTKKRQIYTDIEMNRLGK

SEQ ID NO: 14 - protein, 422 aa, Vesicular Stomatitis Virus
MSVTVKRIIDNTVIVPKLPANEDPVEYPADYFRKSKEIPLYINTTKSLSDLRGYVYQGLKSGNVSIIHVNSYLYGALKDIRGKLDKDWSSFGINIGKAGDTIGIFDLVSLKALDGVLPDGVSDASRTSADDKWLPLYLLGLYRVGRTQMPEYRKRLMDGLTNQCKMINEQFEPLVPEGRDIFDVWGNDSNYTKIVAAVDMFFHMFKKHECASFRYGTIVSRFKDCAALATFGHLCKITGMSTEDVTTWILNREVADEMVQMMLPGQEIDKADSYMPYLIDFGLSSKSPYSSVKNPAFHFWGQLTALLLRSTRARNARQPDDIEYTSLTTAGLLYAYAVGSSADLAQQFCVGDSKYTPDDSTGGLTTNAPPQGRDVVEWLGWFEDQNRKPTPDMMQYAKRAVMSLQGLREKTIGKYAKSEFDK

SEQ ID NO: 15 - protein, 422 aa, synthetic construct
MSVTVKRIIDNTVVVPKLPANEDPVEYPADYFRKSKEIPLYINTTKSLSDLRGYVYQGLKSGNVSIIHVNSYLYGALKDIRGKLDKDWSSFGINIGKAGDTIGIFDLVSLKALDGVLPDGVSDASRTSADDKWLPLYLLGLYRVGRTQMPEYRKKLMDGLTNQCKMINEQFEPLVPEGRDIFDVWGNDSNYTKIVAAVDMFFHMFKKHECASFRYGTIVSRFKDCAALATFGHLCKITGMSTEDVTTWILNREVADEMVQMMLPGQEIDKADSYMPYLIDFGLSSKSPYSSVKNPAFHFWGQLTALLLRSTRARNARQPDDIEYTSLTTAGLLYAYAVGSSADLAQQFCVGDNKYTPDDSTGGLTTNAPPQGRDVVEWLGWFEDQNRKPTPDMMQYAKRAVMSLQGLREKTIGKYAKSEFDK

SEQ ID NO: 16 - protein, 265 aa, Vesicular Stomatitis Virus
MDNLTKVREYLKSYSRLDQAVGEIDEIEAQRAEKSNYELFQEDGVEEHTRPSYFQAADDSDTESEPEIEDNQGLYVPDPEAEQVEGFIQGPLDDYADEDVDVVFTSDWKQPELESDEHGKTLRLTLPEGLSGEQKSQWLLTIKAVVQSAKHWNLAECTFEASGEGVIIKKRQITPDVYKVTPVMNTHPYQSEAVSDVWSLSKTSMTFQPKKASLQPLTISLDELFSSRGEFISVGGNGRMSHKEAILLGLRYKKLYNQARVKYSL

SEQ ID NO: 17 - protein, 265 aa, synthetic construct
MDNLTKVREYLKSYSRLDQAVGEIDEIEAQRAEKSNYELFQEDGVEEHTKPSYFQAADDSDTESEPEIEDNQGLYAPDPEAEQVEGFIQGPLDDYADEEVDVVFTSDWKQPELESDEHGKTLRLTSPEGLSGEQKSQWLSTIKAVVQSAKYWNLAECTFEASGEGVIMKERQITPDVYKVTPVMNTHPSQSEAVSDVWSLSKTSMTFQPKKASLQPLTISLDELFSSRGEFISVGGDGRMSHKEAILLGLRYKKLYNQARVKYSL

SEQ ID NO: 18 - protein, 2109 aa, Vesicular Stomatitis Virus
MEVHDFETDEFNDFNEDDYATREFLNPDERMTYLNHADYNLNSPLISDDIDNLIRKFNSLPIPSMWDSKNWDGVLEMLTSCQANPISTSQMHKWMGSWLMSDNHDASQGYSFLHEVDKEAEITFDVVETFIRGWGNKPIEYIKKERWTDSFKILAYLCQKFLDLHKLTLILNAVSEVELLNLARTFKGKVRRSSHGTNICRIRVPSLGPTFISEGWAYFKKLDILMDRNFLLMVKDVIIGRMQTVLSMVCRIDNLFSEQDIFSLLNIYRIGDKIVERQGNFSYDLIKMVEPICNLKLMKLARESRPLVPQFPHFENHIKTSVDEGAKIDRGIRFLHDQIMSVKTVDLTLVIYGSFRHWGHPFIDYYTGLEKLHSQVTMKKDIDVSYAKALASDLARIVLFQQFNDHKKWFVNGDLLPHDHPFKSHVKENTWPTAAQVQDFGDKWHELPLIKCFEIPDLLDPSIIYSDKSHSMNRSEVLKHVRMNPNIPIPSKKVLQTMLDTKATNWKEFLKEIDEKGLDDDDLIIGLKGKERELKLAGRFFSLMSWKLREYFVITEYLIKTHFVPMFKGLTMADDLTAVIKKMLDSSSGQGLKSYEAICIANHIDYEKWNNHQRKLSNGPVFRVMGQFLGYPSLIERTHEFFEKSLIYYNGRPDLMRVHNNTLINSTSQRVCWQGQEGGLEGLRQKGWSILNLLVIQREAKIRNTAVKVLAQGDNQVICTQYKTKKSRNVVELQGALNQMVSNNEKIMTAIKIGTGKLGLLINDDETMQSADYLNYGKIPIFRGVIRGLETKRWSRVTCVTNDQIPTCANIMSSVSTNALTVAHFAENPINAMIQYNYFGTFARLLLMMHDPALRQSLYEVQDKIPGLHSSTFKYAMLYLDPSIGGVSGMSLSRFLIRAFPDPVTESLSFWRFIHVHARSEHLKEMSAVFGNPEIAKFRITHIDKLVEDPTSLNIAMGMSPANLLKTEVKKCLIESRQTIRNQVIKDATIYLYHEEDRLRSFLWSINPLFPRFLSEFKSGTFLGVADGLISLFQNSRTIRNSFKKKYHRELDDLIVRSEVSSLTHLGKLHLRRGSCKMWTCSATHADTLRYKSWGRTVIGTTVPHPLEMLGPQHRKETPCAPCNTSGFNYVSVHCPDGIHDVFSSRGPLPAYLGSKTSESTSILQPWERESKVPLIKRATRLRDAISWFVEPDSKLAMTILSNIHSLTGEEWTKRQHGFKRTGSALHRFSTSRMSHGGFASQSTAALTRLMATTDTMRDLGDQNFDFLFQATLLYAQITTTVARDGWITSCTDHYHIACKSCLRPIEEITLDSSMDYTPPDVSHVLKTWRNGEGSWGQEIKQIYPLEGNWKNLAPAEQSYQVGRCIGFLYGDLAYRKSTHAEDSSLFPLSIQGRIRGRGFLKGLLDGLMRASCCQVIHRRSLAHLKRPANAVYGGLIYLIDKLSVSPPFLSLTRSGPIRDELETIPHKIPTSYPTSNRDMGVIVRNYFKYQCRLIEKGKYRSHYSQLWLFSDVLSIDFIGPFSISTTLLQILYKPFLSGKDKNELRELANLSSLLRSGEGWEDIHVKFFTKDILLCPEEIRHACKFGIAKDNNKDMSYPPWGRESRGTITTIPVYYTTTPYPKMLEMPPRIQNPLLSGIRLGQLPTGAHYKIRSILHGMGIHYRDFLSCGDGSGGMTAALLRENVHSRGIFNSLLELSGSVMRGASPEPPSALETLGGDKSRCVNGETCWEYPSDLCDPRTWDYFLRLKAGLGLQIDLIVMDMEVRDSSTSLKIETNVRNYVHRILDEQGVLIYKTYGTYICESEKNAVTILGPMFKTVDLVQTEFSSSQTSEVYMVCKGLKKLIDEPNPDWSSINESWKNLYAFQSSEQEFARAKKVSTYFTLTGIPSQFIPDPFVNIETMLQIFGVPTGVSHAAALKSSDRPADLLTISLFYMAIISYYNINHIRVGPIPPNPPSDGIAQNVGIAITGISFWLSLMEKDIPLYQQCLAVIQQSFPIRWEAVSVKGGYKQKWSTRGDGLPKDTRISDSLAPIGNWIRSLELVRNQVRLNPFNEILFNQLCRTVDNHLKWSNLRRNTGMIEWINRRISKEDRSILMLKSDLHEENSWRD

SEQ ID NO: 19 - protein, 2109 aa, synthetic construct
MEVHDFETDEFNDFNEDDYATREFLNPDERMTYLNHADYNLNSPLISDDIDNLIRKFNSLPIPSMWDSKNWDGVLEMLTSCQANPIPTSQMHKWMGSWLMSDNHDASQGYSFLHEVDKEAEITFDVVETFIRGWGNKPIEYIKKERWTDSFKILAYLCQKFLDLHKLTLILNAVSEVELLNLARTFKGKVRRSSHGTNICRIRVPSLGPTFISEGWAYFKKLDILMDRNFLLMVKDVIIGRMQTVLSMVCRIDNLFSEQDIFSLLNIYRIGDKIVERQGNFSYDLIKMVEPICNLKLMKLARESRPLVPQFPHFENHIKTSVDEGAKIDRGIRFLHDQIMSVKTVDLTLVIYGSFRHWGHPFIDYYTGLEKLHSQVTMKKDIDVSYAKALASDLARIVLFQQFNDHKKWFVNGDLLPHDHPFKSHVKENTWPTAAQVQDFGDKWHELPLIKCFEIPDLLDPSIIYSDKSHSMNRSEVLKHVRMNPNTPIPSKKVLQTMLDTKATNWKEFLKEIDEKGLDDDDLIIGLKGKERELKLAGRFFSLMSWKLREYFVITEYLIKTHFVPMFKGLTMADDLTAVIKKMLDSSSGQGLKSYEAICIANHIDYEKWNNHQRKLSNGPVFRVMGQFLGYPSLIERTHEFFEKSLIYYNGRPDLMRVHNNTLINSTSQRVCWQGQEGGLEGLRQKGWSILNLLVIQREAKIRNTAVKVLAQGDNQVICTQYKTKKSRNVVELQGALNQMVSNNEKIMTAIKIGTGKLGLLINDDETMQSADYLNYGKIPIFRGVIRGLETKRWSRVTCVTNDQIPTCANIMSSVSTNALTVAHFAENPINAMIQYNYFGTFARLLLMMHDPALRQSLYEVQDKIPGLHSSTFKYAMLYLDPSIGGVSGMSLSRFLIRAFPDPVTESLSFWRFIHVHARSEHLKEMSAVFGNPEIAKFRITHIDKLVEDPTSLNIAMGMSPANLLKTEVKKCLIESRQTIRNQVIKDATIYLYHEEDRLRSFLWSINPLFPRFLSEFKSGTFLGVADGLISLFQNSRTIRNSFKKKYHRELDDLIVRSEVSSLTHLGKLHLRRGSCKMWTCSATHADTLRYKSWGRTVIGTTVPHPLEMLGPQHRKETPCAPCNTSGFNYVSVHCPDGIHDVFSSRGPLPAYLGSKTSESTSILQPWERESKVPLIKRATRLRDAISWFVEPDSKLAMTILSNIHSLTGEEWTKRQHGFKRTGSALHRFSTSRMSHGGFASQSTAALTRLMATTDTMRDLGDQNFDFLFQATLLYAQITTTVARDGWITSCTDHYHIACKSCLRPIEEITLDSSMDYTPPDVSHVLKTWRNGEGSWGQEIKQIYPLEGNWKNLAPAEQSYQVGRCIGFLYGDLAYRKSTHAEDSSLFPLSIQGRIRGRGFLKGLLDGLMRASCCQVIHRRSLAHLKRPANAVYGGLIYLIDKLSVSPPFLSLTRSGPIRDELETIPHKIPTSYPTSNRDMGVIVRNYFKYQCRLIEKGKYRSHYSQLWLFSDVLSIDFIGPFSISTTLLQILYKPFLSGKDKNELRELANLSSLLRSGEGWEDIHVKFFTKDILLCPEEIRHACKFGIAKDNNKDMSYPPWGRESRGTITTIPVYYTTTPYPKMLEMPPRIQNPLLSGIRLGQLPTGAHYKIRSILHGMGIHYRDFLSCGDGSGGMTAALLRENVHSRGIFNSLLELSGSVMRGASPEPPSALETLGGDKSRCVNGETCWEYPSDLCDPRTWDYFLRLKAGLGLQIDLIVMDMEVRDSSTSLKIETNVRNYVHRILDEQGVLIYKTYGTYICESEKNAVTILGPMFKTVDLVQTEFSSSQTSEVYMVCKGLKKLIDEPNPDWSSINESWKNLYAFQSSEQEFARAKKVSTYFTLTGIPSQFIPDPFVNIETMLQIFGVPTGVSHAAALKSSDRPADLLTISLFYMAIISYYNINHIRVGPIPPNPPSDGIAQNVGIAITGISFWLSLMEKDIPLYQQCLAVIQQSFPIRWEAVSVKGGYKQKWSTRGDGLPKDTRISDSLAPIGNWIRSLELVRNQVRLNPFNEILFNQLCRTVDNHLKWSNLRRNTGMIEWINRRISKEDRSILMLKSDLHEENSWRD

SEQ ID NO: 20 - protein, 144 aa, synthetic construct
MWLQSLLLLGTVACSISAPARSPSPSTQPWEHVNAIQEARRLLNLSRDTAAEMNETVEVISEMFDLQEPTCLQTRLELYKQGLRGSLTKLKGPLTMMASHYKQHCPPTPETSCATQIITFESFKENLKDFLLVIPFDCWEPVQE

SEQ ID NO: 21 - protein, 153 aa, synthetic construct
MYRMQLLSCIALSLALVTNSAPTSSSTKKTQLQLEHLLLDLQMILNGINNYKNPKLTRMLTFKFYMPKKATELKHLQCLEEELKPLEEVLNLAQSKNFHLRPRDLISNINVIVLELKGSETTFMCEYADETATIVEFLNRWITFCQSIISTLT

SEQ ID NO: 22 - protein, 253 aa, synthetic construct
MWPPGSASQPPPSPAAATGLHPAARPVSLQCRLSMCPARSLLLVATLVLLDHLSLARNLPVATPDPGMFPCLHHSQNLLRAVSNMLQKARQTLEFYPCTSEEIDHEDITKDKTSTVEACLPLELTKNESCLNSRETSFITNGSCLASRKTSFMMALCLSSIYEDLKMYQVEFKTMNAKLLMDPKRQIFLDQNMLAVIDELMQALNFNSETVPQKSSLEEPDFYKTKIKLCILLHAFRIRAVTIDRVMSYLNAS

SEQ ID NO: 23 - protein, 328 aa, synthetic construct
MCHQQLVISWFSLVFLASPLVAIWELKKDVYVVELDWYPDAPGEMVVLTCDTPEEDGITWTLDQSSEVLGSGKTLTIQVKEFGDAGQYTCHKGGEVLSHSLLLLHKKEDGIWSTDILKDQKEPKNKTFLRCEAKNYSGRFTCWWLTTISTDLTFSVKSSRGSSDPQGVTCGAATLSAERVRGDNKEYEYSVECQEDSACPAAEESLPIEVMVDAVHKLKYENYTSSFFIRDIIKPDPPKNLQLKPLKNSRQVEVSWEYPDTWSTPHSYFSLTFCVQVQGKSKREKKDRVFTDKTSATVICRKNASISVRAQDRYYSSSWSEWASVPCS

SEQ ID NO: 24 - protein, 162 aa, synthetic construct
MRISKPHLRSISIQCYLCLLLNSHFLTEAGIHVFILGCFSAGLPKTEANWVNVISDLKKIEDLIQSMHIDATLYTESDVHPSCKVTAMKCFLLELQVISLESGDASIHDTVENLIILANNSLSSNGNVTESGCKECEELEEKNIKEFLQSFVHIVQMFINTS

SEQ ID NO: 25 - protein, 193 aa, synthetic construct
MAAEPVEDNCINFVAMKFIDNTLYFIAEDDENLESDYFGKLESKLSVIRNLNDQVLFIDQGNRPLFEDMTDSDCRDNAPRTIFIISMYKDSQPRGMAVTISVKCEKISTLSCENKIISFKEMNPPDNIKDTKSDIIFFQRSVPGHDNKMQFESSSYEGYFLACEKERDLFKLILKKEDELGDRSIMFTVQNED

SEQ ID NO: 26 - protein, 233 aa, synthetic construct
MSTESMIRDVELAEEALPKKTGGPQGSRRCLFLSLFSFLIVAGATTLFCLLHFGVIGPQREEFPRDLSLISPLAQAVRSSSRTPSDKPVAHVVANPQAEGQLQWLNRRANALLANGVELRDNQLVVPSEGLYLIYSQVLFKGQGCPSTHVLLTHTISRIAVSYQTKVNLLSAIKSPCQRETPEGAEAKPWYEPIYLGGVFQLEKGDRLSAEINRPDYLDFAESGQVYFGIIAL

SEQ ID NO: 27 - protein, 187 aa, synthetic construct
MTNKCLLQIALLLCFSTTALSMSYNLLGFLQRSSNFQCQKLLWQLNGRLEYCLKDRMNFDIPEEIKQLQQFQKEDAALTIYEMLQNIFAIFRQDSSSTGWNETIVENLLANVYHQINHLKTVLEEKLEKEDFTRGKLMSSLHLKRYYGRILHYLKAKEYSHCAWTIVRVEILRNFYFINRLTGYLRN

SEQ ID NO: 28 - protein, 323 aa, synthetic construct
MPPPRLLFFLLFLTPMEVRPEEPLVVKVEEGDNAVLQCLKGTSDGPTQQLTWSRESPLKPFLKLSLGLPGLGIHMRPLAIWLFIFNVSQQMGGFYLCQPGPPSEKAWQPGWTVNVEGSGELFRWNVSDLGGLGCGLKNRSSEGPSSPSGKLMSPKLYVWAKDRPEIWEGEPPCLPPRDSLNQSLSQDLTMAPGSTLWLSCGVPPDSVSRGPLSWTHVHPKGPKSLLSLELKDDRPARDMWVMETGLLLPRATAQDAGKYYCHRGNLTMSFHLEITARPVLWHWLLRTGGWKVSAVTLAYLIFCLCSLVGILHLQRALVLRRKR

SEQ ID NO: 29 - protein, 77 aa, synthetic construct
MLQMAGQCSQNEYFDSLLHACIPCQLRCSSNTPPLTCQRYCNASVTNSVKGTNAILWTCLGLSLIISLAVFVLMFLL

SEQ ID NO: 30 - protein, 180 aa, synthetic construct
MQAEGRGTGGSTGDADGPGGPGIPDGPGGNAGGPGEAGATGGRGPRGAGAARASGPGGGAPRGPHGGAASGLNGCCRCGARGPESRLLEFYLAMPFATPMEAELARRSLAQDAPPLPVPGVLLKEFTVSGNILTIRLTAADHRQLQLSISSCLQQLSLLMWITQCFLPVFLAQPPSGQRR

SEQ ID NO: 31 - protein, 1125 aa, synthetic construct
MSGHASSTPGGEKETSATQRSSVPSSTEKNAVSMTSSVLSSHSPGSGSSTTQGQDVTLAPATEPASGSAATWGQDVTSVPVTRPALGSTTPPAHDVTSAPDNKPAPGSTAPPAHGVTSAPDTRPAPGSTAPQAHGVTSAPDTRPAPGSTAPPAHGVTSAPDTRPAPGSTAPPAHGVTSAPDTRPAPGSTAPAAHGVTSAPDTRPAPGSTAPQAHGVTSAPDTRPAPGSTAPPAHGVTSAPDTRPAPGSTAPPAHGVTSAPDTRPAPGSTAPPAHGVTSAPESRPAPGSTAPAAHGVTSAPESRPAPGSTAPAAHGVTSAPESRPAPGSTAPPAHGVTSAPDTRPAPGSTAPPAHGVTSAPDTRPAPGSTAPPAHGVTSAPDTRPAPGSTAPPAHGVTSAPDTRPAPGSTAPPAHGVTSAPESRPAPGSTAPPAHGVTSAPESRPAPGSTAPAAHGVTSAPESRPAPGSTAPAAHGVTSAPESRPAPGSTAPRAHGVTSAPDTRPAPGSTAPPAHGVTSAPDTRPAPGSTAPPAHGVTSAPDTRPAPGSTAPPAHGVTSAPDTRPAPGSTAPPAHGVTSAPDTRPAPGSTAPPAHGVTSAPDTRPAPGSTAPPAHGVTSAPDTRPAPGSTAPAAHGVTSAPESRPAPGSTAPAAHGVTSAPESRPAPGSTAPPAHGVTSAPDTRPAPGSTAPPAHGVTSAPDTRPAPGSTAPPAHGVTSAPDTRPAPGSTAPPAHGVTSAPDTRPAPGSTAPPAHGVTSAPDTRPAPGSTAPPAHGVTSAPDTRPAPGSTAPPAHGVTSAPDTRPAPGSTAPPAHGVTSAPDTRPAPGSTAPPAHGVTSAPDTRRAPGSTPAPGSTAPPAHGVTSAPDTRPAPGSTAPPAHGVTSAPDNRPALGSTAPPVHNVTSASGSASGSASTLVHNGTSARATTTPASKSTPFSIPSHHSDTPTTLASHSTKTDASSTHHSTVPPLTSSNHSTSPQLSTGVSFFFLSFHISNLQFNSSLEDPSTDYYQELQRDISEMFLQIYKQGGFLGLSNIKFRPGSVVVQLTLAFREGTINVHDVETQFNQYKTEAASRYNLTISDVSVSDVPFPFSAQSGAGVPGWGIALLVLVCVLVALAIVYLIAL

SEQ ID NO: 32 - protein, 336 aa, synthetic construct
MEVEKTACPSGKKAREIDESLIFYKKWELEACVDAALLATQMDRVNAIPFTYEQLDVLKHKLDELYPQGYPESVIQHLGYLFLKMSPEDIRKWNVTSLETLKALLEVDKGHEMSPQAPRRPLPQVATLIDRFVKGRGQLDKDTLDTLTAFYPGYLCSLSPEELSSVPPSSIWAVRPQDLDTCDPRQLDVLYPKARLAFQNMNGSEYFVKIQSFLGGAPTEDLKALSQQNVSMDLATFMKLRTDAVLPLTVAEVQKLLGPHVEGLKAEERHRPVRDWILRQRQDDLDTLGLGLQGGIPNGYLVLDLSVQETLSGTPCLLGPGPVLTVLALLLASTLA

SEQ ID NO: 33 - protein, 668 aa, synthetic construct
MRPSGTAGAALLALLAALCPASRALEEKKVCQGTSNKLTQLGTFEDHFLSLQRMFNNCEVVLGNLEITYVQRNYDLSFLKTIQEVAGYVLIALNTVERIPLENLQIIRGNMYYENSYALAVLSNYDANKTGLKELPMRNLQEILHGAVRFSNNPALCNVESIQWRDIVSSDFLSNMSMDFQNHLGSCQKCDPSCPNGSCWGAGEENCQKLTKIICAQQCSGRCRGKSPSDCCHNQCAAGCTGPRESDCLVCRKFRDEATCKDTCPPLMLYNPTTYQMDVNPEGKYSFGATCVKKCPRNYVVTDHGSCVRACGADSYEMEEDGVRKCKKCEGPCRKVCNGIGIGEFKDSLSINATNIKHFKNCTSISGDLHILPVAFRGDSFTHTPPLDPQELDILKTVKEITGFLLIQAWPENRTDLHAFENLEIIRGRTKQHGQFSLAVVSLNITSLGLRSLKEISDGDVIISGNKNLCYANTINWKKLFGTSGQKTKIISNRGENSCKATGQVCHALCSPEGCWGPEPRDCVSCRNVSRGRECVDKCNLLEGEPREFVENSECIQCHPECLPQAMNITCTGRGPDNCIQCAHYIDGPHCVKTCPAGVMGENNTLVWKYADAGHVCHLCHPNCTYGCTGPGLEGCPTNGPKIPSIATGMVGALLLLLVVALGIGLFM

SEQ ID NO: 34 - protein, 785 aa, synthetic construct
MQSKVLLAVALWLCVETRAASVGLPSVSLDLPRLSIQKDILTIKANTTLQITCRGQRDLDWLWPNNQSGSEQRVEVTECSDGLFCKTLTIPKVIGNDTGAYKCFYRETDLASVIYVYVQDYRSPFIASVSDQHGVVYITENKNKTVVIPCLGSISNLNVSLCARYPEKRFVPDGNRISWDSKKGFTIPSYMISYAGMVFCEAKINDESYQSIMYIVVVVGYRIYDVVLSPSHGIELSVGEKLVLNCTARTELNVGIDFNWEYPSSKHQHKKLVNRDLKTQSGSEMKKFLSTLTIDGVTRSDQGLYTCAASSGLMTKKNSTFVRVHEKPFVAFGSGMESLVEATVGERVRIPAKYLGYPPPEIKWYKNGIPLESNHTIKAGHVLTIMEVSERDTGNYTVILTNPISKEKQSHVVSLVVYVPPQIGEKSLISPVDSYQYGTTQTLTCTVYAIPPPHHIHWYWQLEEECANEPSQAVSVTNPYPCEEWRSVEDFQGGNKIEVNKNQFALIEGKNKTVSTLVIQAANVSALYKCEAVNKVGRGERVISFHVTRGPEITLQPDMQPTEQESVSLWCTADRSTFENLTWYKLGPQPLPIHVGELPTPVCKNLDTLWKLNATMFSNSTNDILIMELKNASLQDQGDYVCLAQDRKTKKRHCVVRQLTVLERVAPTITGNLENQTTSIGESIEVSCTASGNPPPQIMWFKDNETLVEDSGIVLKDGNRNLTIRRVRKEDEGLYTCQACSVLGCAKVEAFFIIEGAQEKTNLEIIILVGTAVIAMFFWLLLVII

SEQ ID NO: 35 - protein, 317 aa, synthetic construct
MSSEQKSQHCKPEEGVEAQEEALGLVGAQAPTTEEQEAAVSSSSPLVPGTLEEVPAAESAGPPQSPQGASALPTTISFTCWRQPNEGSSSQEEEGPSTSPDAESLFREALSNKVDELAHFLLRKYRAKELVTKAEMLERVIKNYKRCFPVIFGKASESLKMIFGIDVKEVDPASNTYTLVTCLGLSYDGLLGNNQIFPKTGLLIIVLGTIAMEGDSASEEEIWEELGVMGVYDGREHTVYGEPRKLLTQDWVQENYLEYRQVPGSNPARYEFLWGPRALAETSYVKVLEHVVRVNARVRIAYPSLREAALLEEEEGV

SEQ ID NO: 36 - protein, 931 aa, synthetic construct
ECKEALAKSEMNVNMKYQLPNFTAETPIQNVILHEHHIFLGATNYIYVLNEEDLQKVAEYKTGPVLEHPDCFPCQDCSSKANLSGGVWKDNINMALVVDTYYDDQLISCGSVNRGTCQRHVFPHNHTADIQSEVHCIFSPQIEEPSQCPDCVVSALGAKVLSSVKDRFINFFVGNTINSSYFPDHPLHSISVRRLKETKDGFMFLTDQSYIDVLPEFRDSYPIKYVHAFESNNFIYFLTVQRETLDAQTFHTRIIRFCSINSGLHSYMEMPLECILTEKRKKRSTKKEVFNILQAAYVSKPGAQLARQIGASLNDDILFGVFAQSKPDSAEPMDRSAMCAFPIKYVNDFFNKIVNKNNVRCLQHFYGPNHEHCFNRTLLRNSSGCEARRDEYRTEFTTALQRVDLFMGQFSEVLLTSISTFIKGDLTIANLGTSEGRFMQVVVSRSGPSTPHVNFLLDSHPVSPEVIVEHTLNQNGYTLVITGKKITKIPLNGLGCRHFQSCSQCLSAPPFVQCGWCHDKCVRSEECLSGTWTQQICLPAIYKVFPNSAPLEGGTRLTICGWDFGFRRNNKFDLKKTRVLLGNESCTLTLSESTMNTLKCTVGPAMNKHFNMSIIISNGHGTTQYSTFSYVDPVITSISPKYGPMAGGTLLTLTGNYLNSGNSRHISIGGKTCTLKSVSNSILECYTPAQTISTEFAVKLKIDLANRETSIFSYREDPIVYEIHPTKSFISGGSTITGVGKNLNSVSVPRMVINVHEAGRNFTVACQHRSNSEIICCTTPSLQQLNLQLPLKTKAFFMLDGILSKYFDLIYVHNPVFKPFEKPVMISMGNENVLEIKGNDIDPEAVKGEVLKVGNKSCENIHLHSEAVLCTVPNDLLKLNSELNIEWKQAISSTVLGKVIVQPDQNFTGLIAGVVSISTALLLLLGFFLWL

SEQ ID NO: 37 - protein, 121 aa, synthetic construct
MDQWSTQDLYNNPVTAVFNYQGLWRSCVRESSGFTECRGYFTLLGLPAMLQAVRGGGGSGGGGSGGGGSVTNFWMSTANMYTGMGGMVQTVQTRYTFGAALFVGWVAGGLTLIGGVMMCIA

SEQ ID NO: 38 - protein, 706 aa, synthetic construct
MHLLGPWLLLLVLEYLAFSDSSKWVFEHPETLYAWEGACVWIPCTYRALDGDLESFILFHNPEYNKNTSKFDGTRLYESTKDGKVPSEQKRVQFLGDKNKNCTLSIHPVHLNDSGQLGLRMESKTEKWMERIHLNVSERPFPPHIQLPPEIQESQEVTLTCLLNFSCYGYPIQLQWLLEGVPMRQAAVTSTSLTIKSVFTRSELKFSPQWSHHGKIVTCQLQDADGKFLSNDTVQLNVKHTPKLEIKVTPSDAIVREGDSVTMTCEVSSSNPEYTTVSWLKDGTSLKKQNTFTLNLREVTKDQSGKYCCQVSNDVGPGRSEEVFLQVQYAPEPSTVQILHSPAVEGSQVEFLCMSLANPLPTNYTWYHNGKEMQGRTEEKVHIPKILPWHAGTYSCVAENILGTGQRGPGAELDVQYPPKKVTTVIQNPMPIREGDTVTLSCNYNSSNPSVTRYEWKPHGAWEEPSLGVLKIQNVGWDNTTIACAACNSWCSWASPVALNVQYAPRDVRVRKIKPLSEIHSGNSVSLQCDFSSSHPKEVQFFWEKNGRLLGKESQLNFDSISPEDAGSYSCWVNNSIGQTASKAWTLEVLYAPRRLRVSMSPGDQVMEGKSATLTCESDANPPVSHYTWFDWNNQSLPYHSQKLRLEPVKVQHSGAYWCQGTNSVGKGRSPLSTLTVYYSPETIGRRVAVGLGSCLAILILAICGL

SEQ ID NO: 39 - protein, 295 aa, synthetic construct
MPEEPLVVKVEEGDNAVLQCLKGTSDGPTQQLTWSRESPLKPFLKLSLGLPGLGIHMRPLAIWLFIFNVSQQMGGFYLCQPGPPSEKAWQPGWTVNVEGSGELFRWNVSDLGGLGCGLKNRSSEGPSSPSGKLMSPKLYVWAKDRPEIWEGEPPCLPPRDSLNQSLSQDLTMAPGSTLWLSCGVPPDSVSRGPLSWTHVHPKGPKSLLSLELKDDRPARDMWVMETGLLLPRATAQDAGKYYCHRGNLTMSFHLEITARPVLWHWLLRTGGWKVSAVTLAYLIFCLCSLVGILHL

SEQ ID NO: 40 - protein, 317 aa, synthetic construct
MSSEQKSQHCKPEEGVEAQEEALGLVGAQAPTTEEQEAAVSSSSPLVPGTLEEVPAAESAGPPQSPQGASALPTTISFTCWRQPNEGSSSQEEEGPSTSPDAESLFREALSNKVDELAHFLLRKYRAKELVTKAEMLERVIKNYKRCFPVIFGKASESLKMIFGIDVKEVDPTSNTYTLVTCLGLSYDGLLGNNQIFPKTGLLIIVLGTIAMEGDSASEEEIWEELGVMGVYDGREHTVYGEPRKLLTQDWVQENYLEYRQVPGSNPARYEFLWGPRALAETSYVKVLEHVVRVNARVRIAYPSLREAALLEEEEGV

SEQ ID NO: 41 - protein, 169 aa, synthetic construct
MDQWSTQDLYNNPVTAVFNYQGLWRSCVRESSGFTECRGYFTLLGLPAMLQAVRALMIVGIVLGAIGLLVSIFALKCIRIGSMEDSAKANMTLTSGIMFIVSGLCAIAGVSVFANMLVTNFWMSTANMYTGMGGMVQTVQTRYTFGAALFVGWVAGGLTLIGGVMMCIA